European Patent Application EP 4 144 757 A1, published March 8, 2023. Title: Long-acting dual agonists of GLP-1/glucagon receptors. Applicant: DONG-A ST CO., LTD. The sequence listing filed with the application follows.

SEQUENCE LISTING (14 sequences)

SEQ ID NO: 1 - protein, 37 aa, Homo sapiens
HSQGTFTSDKSKYLDSRRAQDFVQWLMNTKRNRNNIA

SEQ ID NO: 2 - protein, 37 aa, Artificial Sequence
  oxyntomodulin analogue
  MOD_RES (2): Xaa=aminoisobutyric acid
  MOD_RES (10): Lys=([(2-(2-(2-aminoethoxy)ethoxy)acetoyl)2]-[gammaglutamyl]-[oct adecanoyl])
  MOD_RES (16): Xaa=aminoisobutyric acid
  MOD_RES (34): Lys=(13-carboxy-1-oxotridecyl)
HXQGTFTSDKSKYLDXRRAQDFVQWLMNTKEYEKEYE

SEQ ID NO: 3 - protein, 37 aa, Artificial Sequence; identical to SEQ ID NO: 2
  oxyntomodulin analogue
  MOD_RES (2): Xaa=aminoisobutyric acid
  MOD_RES (10): Lys=([(2-(2-(2-aminoethoxy)ethoxy)acetoyl)2]-[gammaglutamyl]-[oct adecanoyl])
  MOD_RES (16): Xaa=aminoisobutyric acid
  MOD_RES (34): Lys=(15-carboxy-1-oxopentadecyl)

SEQ ID NO: 4 - protein, 37 aa, Artificial Sequence; identical to SEQ ID NO: 2
  oxyntomodulin analogue
  MOD_RES (2): Xaa=aminoisobutyric acid
  MOD_RES (10): Lys=([(2-(2-(2-aminoethoxy)ethoxy)acetoyl)2]-[gammaglutamyl]-[oct adecanoyl])
  MOD_RES (16): Xaa=aminoisobutyric acid
  MOD_RES (34): Lys=(17-carboxy-1-oxoheptadecyl)

SEQ ID NO: 5 - protein, 37 aa, Artificial Sequence; identical to SEQ ID NO: 2
  oxyntomodulin analogue
  MOD_RES (2): Xaa=aminoisobutyric acid
  MOD_RES (10): Lys=([(2-(2-(2-aminoethoxy)ethoxy)acetoyl)2]-[gammaglutamyl]-[oct adecanoyl])
  MOD_RES (16): Xaa=aminoisobutyric acid
  MOD_RES (34): Lys=([lysyl]-[17-carboxy-1-oxoheptadecyl])

SEQ ID NO: 6 - protein, 37 aa, Artificial Sequence; identical to SEQ ID NO: 2
  oxyntomodulin analogue
  MOD_RES (2): Xaa=aminoisobutyric acid
  MOD_RES (10): Lys=([(2-(2-(2-aminoethoxy)ethoxy)acetoyl)2]-[gammaglutamyl]-[oct adecanoyl])
  MOD_RES (16): Xaa=aminoisobutyric acid
  MOD_RES (34): Lys=([(2-(2-(2-aminoethoxy)ethoxy)acetoyl)3]-[gammaglutamyl]-[17- carboxy-1-oxoheptadecyl])

SEQ ID NO: 7 - protein, 37 aa, Artificial Sequence; identical to SEQ ID NO: 2
  oxyntomodulin analogue
  MOD_RES (2): Xaa=aminoisobutyric acid
  MOD_RES (10): Lys=([(2-(2-(2-aminoethoxy)ethoxy)acetoyl)2]-[gammaglutamyl]-[oct adecanoyl])
  MOD_RES (16): Xaa=aminoisobutyric acid
  MOD_RES (34): Lys=([lysyl]-[(2-(2-(2-aminoethoxy)ethoxy)acetoyl)3]-[gammaglutam yl]-[17-carboxy-1-oxoheptadecyl])

SEQ ID NO: 8 - protein, 37 aa, Artificial Sequence; identical to SEQ ID NO: 2
  oxyntomodulin analogue
  MOD_RES (2): Xaa=aminoisobutyric acid
  MOD_RES (10): Lys=([(2-(2-(2-aminoethoxy)ethoxy)acetoyl)2]-[gammaglutamyl]-[oct adecanoyl])
  MOD_RES (16): Xaa=aminoisobutyric acid
  MOD_RES (34): Lys=(17-aminocarboxy-1-oxoheptadecyl)

SEQ ID NO: 9 - protein, 30 aa, Artificial Sequence
  oxyntomodulin analogue
  MOD_RES (2): Xaa=aminoisobutyric acid
  MOD_RES (10): Lys=([(2-(2-(2-aminoethoxy)ethoxy)acetoyl)2]-[gammaglutamyl]-[oct adecanoyl])
  MOD_RES (16): Xaa=aminoisobutyric acid
HXQGTFTSDKSKYLDXRRAQDFVQWLMNTK

SEQ ID NO: 10 - protein, 37 aa, Artificial Sequence; identical to SEQ ID NO: 2
  oxyntomodulin analogue
  MOD_RES (2): Xaa=aminoisobutyric acid
  MOD_RES (10): Lys=([(2-(2-(2-aminoethoxy)ethoxy)acetoyl)2]-[gammaglutamyl]-[oct adecanoyl])
  MOD_RES (16): Xaa=aminoisobutyric acid
  MOD_RES (34): Lys=(hexadecanoyl)

SEQ ID NO: 11 - protein, 37 aa, Artificial Sequence; identical to SEQ ID NO: 2
  oxyntomodulin analogue
  MOD_RES (2): Xaa=aminoisobutyric acid
  MOD_RES (10): Lys=([(2-(2-(2-aminoethoxy)ethoxy)acetoyl)2]-[gammaglutamyl]-[oct adecanoyl])
  MOD_RES (16): Xaa=aminoisobutyric acid
  MOD_RES (34): Lys=(13-aminocarboxy-1-oxotridecyl)

SEQ ID NO: 12 - protein, 37 aa, Artificial Sequence; identical to SEQ ID NO: 2
  oxyntomodulin analogue
  MOD_RES (2): Xaa=aminoisobutyric acid
  MOD_RES (10): Lys=([(2-(2-(2-aminoethoxy)ethoxy)acetoyl)2]-[gammaglutamyl]-[oct adecanoyl])
  MOD_RES (16): Xaa=aminoisobutyric acid
  MOD_RES (34): Lys=(15-aminocarboxy-1-oxopentadecyl)

SEQ ID NO: 13 - protein, 37 aa, Artificial Sequence; identical to SEQ ID NO: 2
  oxyntomodulin analogue
  MOD_RES (2): Xaa=aminoisobutyric acid
  MOD_RES (10): Lys=([(2-(2-(2-aminoethoxy)ethoxy)acetoyl)2]-[gammaglutamyl]-[oct adecanoyl])
  MOD_RES (16): Xaa=aminoisobutyric acid
  MOD_RES (34): Lys=([(2-(2-(2-aminoethoxy)ethoxy)acetoyl)3]-[hexadecanoyl])

SEQ ID NO: 14 - protein, 37 aa, Artificial Sequence
  oxyntomodulin analogue
  MOD_RES (2): Xaa=aminoisobutyric acid
  VARIANT (10): Xaa=Lys
  MOD_RES (16): Xaa=aminoisobutyric acid
  VARIANT (34): Xaa=Lys
HXQGTFTSDXSKYLDXRRAQDFVQWLMNTKEYEXEYE